European Patent Specification EP 3 221 351 B1, published November 13, 2024. Title: METHODS AND COMPOSITIONS FOR CANCER TREATMENT USING A SINGLE-CHAIN ANTI-EPHA2 ANTIBODY. Applicant: NIKOLOV, Dimitar B. HIMANEN, Juha. The sequence listing filed with the application follows.

SEQUENCE LISTING (9 sequences)

SEQ ID NO: 1 - protein, 253 aa, Artificial Sequence
  Synthetic
EIVLTQSPGTLSLSPGERATLSCRASQSVSSSNLAWYQQKPGQAPRLLIYGASSRATGVPDRFSGSGSGTDFTLTISRLEPEDFAVYYCQQSSSYPWTFGQGTKVEIKRTGGGGSGAGGSGGGGTGGGGSEVQLLESGGGLVQPGGSLRLSCAASGFTFSRYWMHWVRQAPGKGLEWVSSISPYDGETNYADSVKGRFTISRDNSKNTLYLQMNSLRAEDTAVYYCARISEWYNWAVDVFDYWGQGTLVTVSS

SEQ ID NO: 2 - DNA, 1565 bp, Artificial Sequence
  Synthetic
aaaagcggcccagccggccatggcgcaaattgttctctcccagtctccagcaatcctgtctgcatctccaggggagaaggtcacaatgacttgcagggccagctcaagtgtaagttacatacactggttccagcagaagccaggatcctcccccaaaccctggatttatgccacatccaacctggcttctggagtccctgtacgcttcagtggcagtgggtctgggacctcttactctctcacaatcagcagagtggaggctgaagatgctgccacttattactgccagcagtggacaagtaacccaccgacgttcggtggaggcaccaagctggaaatcaaacgcacaggtggtggcggcagtggcgccggtgggtctggaggtggcggtaccggtggcggagggtcacaggtgcagctgcagcagcccggcgctgaactagtaaaaccgggcgcttcagtgaaaatgtcctgcaaagcatccggctacaccttcacctcatacaatatgcactgggtaaaacagacaccgggccgaggcctggaatggatcggcgcaatctacccgggcaacggcgacacctcatacaaccaaaaattcaaaggcaaagcaaccctcaccgcagacaaatcctcatccacagcttacatgcaactgtcctccctgacatccgaagactcagcagtgtactactgcgctcgctccacatactatggaggcgactggtacttcaacgtgtggggcgcaggcaccacagtgaccgtgtccgctggtggtggcggcagtggcgagatcgtgctgacccaatctccgggcacactgagcttgtctccgggcgaacgtgcgacccttagctgcagagccagccagtcggtgtccagctcgaaccttgcgtggtatcaacagaaaccaggtcaagcacctcgcctgctgatttatggcgcctcttcacgtgccactggggtcccggatcgctttagcggctctggcagtggcaccgattttactctgaccatttcccgtctggaaccggaagacttcgcggtgtactattgtcagcagtcctccagctatccttggacctttggccaggggacgaaagtcgagattaaacgcacaggtggtggcggcagtggcgccggtgggtctggaggtggcggtaccggtggcggagggtcagaggtacagctgcttgaaagcggcggtggcctggtgcaaccgggtgggagcctgcgtctgtcgtgcgcagcctccggatttacgttctcccgttactggatgcactgggtccgtcaggctccaggtaagggtctcgagtgggtcagttctatctctccgtacgacggggaaacgaactatgcagatagcgtgaagggtcgcttcaccatctcccgggacaattcgaagaacacactgtatctccaaatgaactcgcttcgtgctgaggacactgccgtctactactgtgctcgtatctctgaatggtacaactgggctgttgacgttttcgactactggggtcagggtacactagtcaccgtgagctcggcctcgggggccaaaa

SEQ ID NO: 3 - protein, 249 aa, Artificial Sequence
  Synthetic
QIVLSQSPAILSASPGEKVTMTCRASSSVSYIHWFQQKPGSSPKPWIYATSNLASGVPVRFSGSGSGTSYSLTISRVEAEDAATYYCQQWTSNPPTFGGGTKLEIKRTGGGGSGAGGSGGGGTGGGGSQVQLQQPGAELVKPGASVKMSCKASGYTFTSYNMHWVKQTPGRGLEWIGAIYPGNGDTSYNQKFKGKATLTADKSSSTAYMQLSSLTSEDSAVYYCARSTYYGGDWYFNVWGAGTTVTVSA

SEQ ID NO: 4 - protein, 521 aa, Artificial Sequence
  Synthetic
KAAQPAMAQIVLSQSPAILSASPGEKVTMTCRASSSVSYIHWFQQKPGSSPKPWIYATSNLASGVPVRFSGSGSGTSYSLTISRVEAEDAATYYCQQWTSNPPTFGGGTKLEIKRTGGGGSGAGGSGGGGTGGGGSQVQLQQPGAELVKPGASVKMSCKASGYTFTSYNMHWVKQTPGRGLEWIGAIYPGNGDTSYNQKFKGKATLTADKSSSTAYMQLSSLTSEDSAVYYCARSTYYGGDWYFNVWGAGTTVTVSAGGGGSGEIVLTQSPGTLSLSPGERATLSCRASQSVSSSNLAWYQQKPGQAPRLLIYGASSRATGVPDRFSGSGSGTDFTLTISRLEPEDFAVYYCQQSSSYPWTFGQGTKVEIKRTGGGGSGAGGSGGGGTGGGGSEVQLLESGGGLVQPGGSLRLSCAASGFTFSRYWMHWVRQAPGKGLEWVSSISPYDGETNYADSVKGRFTISRDNSKNTLYLQMNSLRAEDTAVYYCARISEWYNWAVDVFDYWGQGTLVTVSSASGAK

SEQ ID NO: 5 - protein, 246 aa, Artificial Sequence
  Synthetic
EIVLTQSPGTLSLSPGERATLSCRASQSVSSSYLHWYQQKPGQAPRLLIYGASSRATGVPDRFSGSGSGTDFTLTISRLEPEDFAVYYCQQHYSIPSTFGQGTKVEIKRTGGGGSGAGGSGGGGTGGGGSEVQLLESGGGLVQPGGSLRLSCAASGFTFSSYLMHWVRQAPGKGLEWVSLITPSGGSTHYADSVKGRFTISRDNSKNTLYLQMNSLRAEDTAVYYCARSGFGYWGQGTLVTVSSAS

SEQ ID NO: 6 - protein, 248 aa, Artificial Sequence
  Synthetic
EIVLTQSPGTLSLSPGERATLSCRASQSVSSSTLNWYQQKPGQAPRLLIYGASSRATGVPDRFSGSGSGTDFTLTISRLEPEDFAVYYCHQDNSNPRTFGQGTKVEIKRTGGGGSGAGGSGGGGTGGGGSEVQLLESGGGLVQPGGSLRLSCAASGFTFSSYLMNWVRQAPGKGLEWVSEINPSGGSTYYADSVKGRFTISRDNSKNTLYLQMNSLRAEDTAVYYCASWGPWFDYWGQGTLVTVSSAS

SEQ ID NO: 7 - protein, 248 aa, Artificial Sequence
  Synthetic
EIVLTQSPGTLSLSPGERATLSCRASQSVSSSSLNWYQQKPGQAPRLLIYGASSRATGVPDRFSGSGSGTDFTLTISRLEPEDFAVYYCLQRYYSPRTFGQGTKVEIKRTGGGGSGAGGSGGGGTGGGGSEVQLLESGGGLVQPGGSLRLSCAASGFTFSSYLMSWVRQAPGKGLEWVSSIDSSGGSTYYADSVKGRFTISRDNSKNTLYLQMNSLRAEDTAVYYCGRSTPLGDYWGQGTLVTVSSAS

SEQ ID NO: 8 - DNA, 1524 bp, Artificial Sequence
  Synthetic
caaattgttctctcccagtctccagcaatcctgtctgcatctccaggggagaaggtcacaatgacttgcagggccagctcaagtgtaagttacatacactggttccagcagaagccaggatcctcccccaaaccctggatttatgccacatccaacctggcttctggagtccctgtacgcttcagtggcagtgggtctgggacctcttactctctcacaatcagcagagtggaggctgaagatgctgccacttattactgccagcagtggacaagtaacccaccgacgttcggtggaggcaccaagctggaaatcaaacgcacaggtggtggcggcagtggcgccggtgggtctggaggtggcggtaccggtggcggagggtcacaggtgcagctgcagcagcccggcgctgaactagtaaaaccgggcgcttcagtgaaaatgtcctgcaaagcatccggctacaccttcacctcatacaatatgcactgggtaaaacagacaccgggccgaggcctggaatggatcggcgcaatctacccgggcaacggcgacacctcatacaaccaaaaattcaaaggcaaagcaaccctcaccgcagacaaatcctcatccacagcttacatgcaactgtcctccctgacatccgaagactcagcagtgtactactgcgctcgctccacatactatggaggcgactggtacttcaacgtgtggggcgcaggcaccacagtgaccgtgtccgctggtggtggcggcagtggcgagatcgtgctgacccaatctccgggcacactgagcttgtctccgggcgaacgtgcgacccttagctgcagagccagccagtcggtgtccagctcgaaccttgcgtggtatcaacagaaaccaggtcaagcacctcgcctgctgatttatggcgcctcttcacgtgccactggggtcccggatcgctttagcggctctggcagtggcaccgattttactctgaccatttcccgtctggaaccggaagacttcgcggtgtactattgtcagcagtcctccagctatccttggacctttggccaggggacgaaagtcgagattaaacgcacaggtggtggcggcagtggcgccggtgggtctggaggtggcggtaccggtggcggagggtcagaggtacagctgcttgaaagcggcggtggcctggtgcaaccgggtgggagcctgcgtctgtcgtgcgcagcctccggatttacgttctcccgttactggatgcactgggtccgtcaggctccaggtaagggtctcgagtgggtcagttctatctctccgtacgacggggaaacgaactatgcagatagcgtgaagggtcgcttcaccatctcccgggacaattcgaagaacacactgtatctccaaatgaactcgcttcgtgctgaggacactgccgtctactactgtgctcgtatctctgaatggtacaactgggctgttgacgttttcgactactggggtcagggtacactagtcaccgtgagctcg

SEQ ID NO: 9 - protein, 508 aa, Artificial Sequence
  Synthetic
QIVLSQSPAILSASPGEKVTMTCRASSSVSYIHWFQQKPGSSPKPWIYATSNLASGVPVRFSGSGSGTSYSLTISRVEAEDAATYYCQQWTSNPPTFGGGTKLEIKRTGGGGSGAGGSGGGGTGGGGSQVQLQQPGAELVKPGASVKMSCKASGYTFTSYNMHWVKQTPGRGLEWIGAIYPGNGDTSYNQKFKGKATLTADKSSSTAYMQLSSLTSEDSAVYYCARSTYYGGDWYFNVWGAGTTVTVSAGGGGSGEIVLTQSPGTLSLSPGERATLSCRASQSVSSSNLAWYQQKPGQAPRLLIYGASSRATGVPDRFSGSGSGTDFTLTISRLEPEDFAVYYCQQSSSYPWTFGQGTKVEIKRTGGGGSGAGGSGGGGTGGGGSEVQLLESGGGLVQPGGSLRLSCAASGFTFSRYWMHWVRQAPGKGLEWVSSISPYDGETNYADSVKGRFTISRDNSKNTLYLQMNSLRAEDTAVYYCARISEWYNWAVDVFDYWGQGTLVTVSS